European Patent Specification EP 4 025 598 B1, published July 8, 2026. Title: Proteins Comprising T-Cell Receptor Constant Domains. Applicant: Eli Lilly and Company The University of North Carolina at Chapel Hill. The sequence listing filed with the application follows.

SEQUENCE LISTING (52 sequences)

SEQ ID NO: 1 - protein, 96 aa, Homo sapiens
PYIQNPDPAVYQLRDSKSSDKSVCLFTDFDSQTNVSQSKDSDVYITDKTVLDMRSMDFKSNSAVAWSNKSDFACANAFNNSIIPEDTFFPSPESSC

SEQ ID NO: 2 - protein, 131 aa, Homo sapiens
EDLKNVFPPEVAVFEPSEAEISHTQKATLVCLATGFYPDHVELSWWVNGKEVHSGVSTDPQPLKEQPALNDSRYALSSRLRVSATFWQDPRNHFRCQVQFYGLSENDEWTQDRAKPVTQIVSAEAWGRADC

SEQ ID NO: 3 - protein, 96 aa, Artificial Sequence
  Synthetic Construct
PYIQNPDPAVYQLRDSKSSDKSVCLFTDFDSQTNVSQSKDSDVYITDKCVLDMRSMDFKSNSAVAWSNKSDFACANAFNNSIIPEDTFFPSPESSC

SEQ ID NO: 4 - protein, 131 aa, Artificial Sequence
  Synthetic Construct
EDLKNVFPPEVAVFEPSEAEISHTQKATLVCLATGFYPDHVELSWWVNGKEVHSGVCTDPQPLKEQPALNDSRYALSSRLRVSATFWQDPRNHFRCQVQFYGLSENDEWTQDRAKPVTQIVSAEAWGRADC

SEQ ID NO: 5 - protein, 96 aa, Artificial Sequence
  Synthetic Construct
PYIQNPDPAVYQLRDSKSSDKFVCLFTDFDSQINVSQSKDSDVYITDKTVLDMRSMDFKSNSAVAWSNKSDFTCANAFNNSIIPEDTFFPSPESSC

SEQ ID NO: 6 - protein, 96 aa, Artificial Sequence
  Synthetic Construct
PYIQNPDPAVYQLRDSKSSDKFVCLFTDFDSQINVSQSKDSDVYITDKCVLDMRSMDFKSNSAVAWSNKSDFTCANAFNNSIIPEDTFFPSPESSC

SEQ ID NO: 7 - protein, 131 aa, Artificial Sequence
  Synthetic Construct
EDLKNVFPPEVAVFEPSKAEISRTQKATLVCLATGFYPPHVELSWWVNGKEVHDGVSTDPQPLKEQPALNDSRYALSSRLRVSATFWQDPRNHFRCQVQFYGLSENDEWTQDRAKPVTQIVSAEAWGRADC

SEQ ID NO: 8 - protein, 131 aa, Artificial Sequence
  Synthetic Construct
EDLKNVFPPEVAVFEPSKAEISRTQKATLVCLATGFYPPHVELSWWVNGKEVHDGVCTDPQPLKEQPALNDSRYALSSRLRVSATFWQDPRNHFRCQVQFYGLSENDEWTQDRAKPVTQIVSAEAWGRADC

SEQ ID NO: 9 - protein, 208 aa, Homo sapiens
QEVTQIPAALSVPEGENLVLNCSFTDSAIYNLQWFRQDPGKGLTSLLLISPWQREQTSGRLNASLDKSSGRSTLYIAASQPGDSATYLCAVRPLLDGTYIPTFGRGTSLIVHPYIQNPDPAVYQLRDSKSSDKSVCLFTDFDSQTNVSQSKDSDVYITDKTVLDMRSMDFKSNSAVAWSNKSDFTCANAFNNSIIPEDTFFPSPESSC

SEQ ID NO: 10 - protein, 208 aa, Artificial Sequence
  Synthetic Construct
QEVTQIPAALSVPEGENLVLNCSFTDSAIYNLQWFRQDPGKGLTSLLLISPWQREQTSGRLNASLDKSSGRSTLYIAASQPGDSATYLCAVRPLLDGTYIPTFGRGTSLIVHPYIQNPDPAVYQLRDSKSSDKSVCLFTDFDSQTNVSQSKDSDVYITDKCVLDMRSMDFKSNSAVAWSNKSDFTCANAFNNSIIPEDTFFPSPESSC

SEQ ID NO: 11 - protein, 208 aa, Artificial Sequence
  Synthetic Construct
QEVTQIPAALSVPEGENLVLNCSFTDSAIYNLQWFRQDPGKGLTSLLLISPWQREQTSGRLNASLDKSSGRSTLYIAASQPGDSATYLCAVRPLLDGTYIPTFGRGTSLIVHPYIQNPDPAVYQLRDSKSSDKFVCLFTDFDSQINVSQSKDSDVYITDKCVLDMRSMDFKSNSAVAWSNKSDFTCANAFNNSIIPEDTFFPSPESSC

SEQ ID NO: 12 - protein, 208 aa, Artificial Sequence
  Synthetic Construct
QEVTQIPAALSVPEGENLVLNCSFTDSAIYNLQWFRQDPGKGLTSLLLISPWQREQTSGRLNASLDKSSGRSTLYIAASQPGDSATYLCAVRPLLDGTYIPTFGRGTSLIVHPYIQNPDPAVYQLRDSKSSDKFVCLFTDFDSQINVSQSKDSDVYITDKTVLDMRSMDFKSNSAVAWSNKSDFTCANAFNNSIIPEDTFFPSPESSC

SEQ ID NO: 13 - protein, 242 aa, Homo sapiens
GVTQTPKFQVLKTGQSMTLQCAQDMNHEYMSWYRQDPGMGLRLIHYSVAIQTTDQGEVPNGYNVSRSTIEDFPLRLLSAAPSQTSVYFCASSYVGDTGELFFGEGSRLTVLEDLKNVFPPEVAVFEPSEAEISHTQKATLVCLATGFYPDHVELSWWVNGKEVHSGVSTDPQPLKEQPALNDSRYALSSRLRVSATFWQDPRNHFRCQVQFYGLSENDEWTQDRAKPVTQIVSAEAWGRADC

SEQ ID NO: 14 - protein, 242 aa, Artificial Sequence
  Synthetic Construct
GVTQTPKFQVLKTGQSMTLQCAQDMNHEYMSWYRQDPGMGLRLIHYSVAIQTTDQGEVPNGYNVSRSTIEDFPLRLLSAAPSQTSVYFCASSYVGDTGELFFGEGSRLTVLEDLKNVFPPEVAVFEPSEAEISHTQKATLVCLATGFYPDHVELSWWVNGKEVHSGVCTDPQPLKEQPALNDSRYALSSRLRVSATFWQDPRNHFRCQVQFYGLSENDEWTQDRAKPVTQIVSAEAWGRADC

SEQ ID NO: 15 - protein, 242 aa, Artificial Sequence
  Synthetic Construct
GVTQTPKFQVLKTGQSMTLQCAQDMNHEYMSWYRQDPGMGLRLIHYSVAIQTTDQGEVPNGYNVSRSTIEDFPLRLLSAAPSQTSVYFCASSYVGDTGELFFGEGSRLTVLEDLKNVFPPEVAVFEPSKAEISRTQKATLVCLATGFYPPHVELSWWVNGKEVHDGVCTDPQPLKEQPALNDSRYALSSRLRVSATFWQDPRNHFRCQVQFYGLSENDEWTQDRAKPVTQIVSAEAWGRADC

SEQ ID NO: 16 - protein, 242 aa, Artificial Sequence
  Synthetic Construct
GVTQTPKFQVLKTGQSMTLQCAQDMNHEYMSWYRQDPGMGLRLIHYSVAIQTTDQGEVPNGYNVSRSTIEDFPLRLLSAAPSQTSVYFCASSYVGDTGELFFGEGSRLTVLEDLKNVFPPEVAVFEPSKAEISRTQKATLVCLATGFYPPHVELSWWVNGKEVHDGVSTDPQPLKEQPALNDSRYALSSRLRVSATFWQDPRNHFRCQVQFYGLSENDEWTQDRAKPVTQIVSAEAWGRADC

SEQ ID NO: 17 - protein, 205 aa, Artificial Sequence
  Synthetic Construct
QQVKQNSPSLSVQEGRISILNCDYTNSMFDYFLWYKKYPAEGPTFLISISSIKDKNEDGRFTVFLNKSAKHLSLHIVPSQPGDSAVYFCAASGDFNKFYFGSGTKLNVKPYIQNPDPAVYQLRDSKSSDKSVCLFTDFDSQTNVSQSKDSDVYITDKCVLDMRSMDFKSNSAVAWSNKSDFACANAFNNSIIPEDTFFPSPESSC

SEQ ID NO: 18 - protein, 205 aa, Artificial Sequence
  Synthetic Construct
QQVKQNSPSLSVQEGRISILNCDYTNSMFDYFLWYKKYPAEGPTFLISISSIKDKNEDGRFTVFLNKSAKHLSLHIVPSQPGDSAVYFCAASGDFNKFYFGSGTKLNVKPYIQNPDPAVYQLRDSKSSDKFVCLFTDFDSQINVSQSKDSDVYITDKCVLDMRSMDFKSNSAVAWSNKSDFTCANAFNNSIIPEDTFFPSPESSC

SEQ ID NO: 19 - protein, 245 aa, Artificial Sequence
  Synthetic Construct
EAGVAQSPRYKIIEKRQSVAFWCNPISGHATLYWYQQILGQGPKLLIQFQNNGVVDDSQLPKDRFSAERLKGVDSTLKIQPAKLEDSAVYLCASSLGTGLGEQYFGPGTRLTVTEDLKNVFPPEVAVFEPSEAEISHTQKATLVCLATGFYPDHVELSWWVNGKEVHSGVCTDPQPLKEQPALNDSRYALSSRLRVSATFWQDPRNHFRCQVQFYGLSENDEWTQDRAKPVTQIVSAEAWGRADC

SEQ ID NO: 20 - protein, 245 aa, Artificial Sequence
  Synthetic Construct
EAGVAQSPRYKIIEKRQSVAFWCNPISGHATLYWYQQILGQGPKLLIQFQNNGVVDDSQLPKDRFSAERLKGVDSTLKIQPAKLEDSAVYLCASSLGTGLGEQYFGPGTRLTVTEDLKNVFPPEVAVFEPSKAEISRTQKATLVCLATGFYPPHVELSWWVNGKEVHDGVCTDPQPLKEQPALNDSRYALSSRLRVSATFWQDPRNHFRCQVQFYGLSENDEWTQDRAKPVTQIVSAEAWGRADC

SEQ ID NO: 21 - protein, 206 aa, Artificial Sequence
  Synthetic Construct
QQKEVEQNSGPLSVPEGAIASLNCTYSDRGSQSFFWYRQYSGKSPELIMSIYSNGDKEDGRFTAQLNKASQYVSLLIRDSQPSDSATYLWGTYNQGGKLIFGQGTELSVKPYIQNPDPAVYQLRDSKSSDKSVCLFTDFDSQTNVSQSKDSDVYITDKCVLDMRSMDFKSNSAVAWSNKSDFACANAFNNSIIPEDTFFPSPESSC

SEQ ID NO: 22 - protein, 206 aa, Artificial Sequence
  Synthetic Construct
QQKEVEQNSGPLSVPEGAIASLNCTYSDRGSQSFFWYRQYSGKSPELIMSIYSNGDKEDGRFTAQLNKASQYVSLLIRDSQPSDSATYLWGTYNQGGKLIFGQGTELSVKPYIQNPDPAVYQLRDSKSSDKFVCLFTDFDSQINVSQSKDSDVYITDKCVLDMRSMDFKSNSAVAWSNKSDFTCANAFNNSIIPEDTFFPSPESSC

SEQ ID NO: 23 - protein, 240 aa, Artificial Sequence
  Synthetic Construct
QVTQNPRYLITVTGKKLTVTCSQNMNHEYMSWYRQDPGLGLRQIYYSMNVEVTDKGDVPEGYKVSRKEKRNFPLILESPSPNQTSLYFCASSGASHEQYFGPGTRLTVTEDLKNVFPPEVAVFEPSEAEISHTQKATLVCLATGFYPDHVELSWWVNGKEVHSGVCTDPQPLKEQPALNDSRYALSSRLRVSATFWQDPRNHFRCQVQFYGLSENDEWTQDRAKPVTQIVSAEAWGRADC

SEQ ID NO: 24 - protein, 240 aa, Artificial Sequence
  Synthetic Construct
QVTQNPRYLITVTGKKLTVTCSQNMNHEYMSWYRQDPGLGLRQIYYSMNVEVTDKGDVPEGYKVSRKEKRNFPLILESPSPNQTSLYFCASSGASHEQYFGPGTRLTVTEDLKNVFPPEVAVFEPSKAEISRTQKATLVCLATGFYPPHVELSWWVNGKEVHDGVCTDPQPLKEQPALNDSRYALSSRLRVSATFWQDPRNHFRCQVQFYGLSENDEWTQDRAKPVTQIVSAEAWGRADC

SEQ ID NO: 25 - protein, 209 aa, Artificial Sequence
  Synthetic Construct
KQEVTQIPAALSVPEGENLVLNCSFTDSAIYNLQWFRQDPGKGLTSLLYVRPYQREQTSGRLNASLDKSSGRSTLYIAASQPGDSATYLCAVRPGGAGPFFVVFGKGTKLSVIPYIQNPDPAVYQLRDSKSSDKSVCLFTDFDSQTNVSQSKDSDVYITDKCVLDMRSMDFKSNSAVAWSNKSDFACANAFNNSIIPEDTFFPSPESSC

SEQ ID NO: 26 - protein, 209 aa, Artificial Sequence
  Synthetic Construct
KQEVTQIPAALSVPEGENLVLNCSFTDSAIYNLQWFRQDPGKGLTSLLYVRPYQREQTSGRLNASLDKSSGRSTLYIAASQPGDSATYLCAVRPGGAGPFFVVFGKGTKLSVIPYIQNPDPAVYQLRDSKSSDKFVCLFTDFDSQINVSQSKDSDVYITDKCVLDMRSMDFKSNSAVAWSNKSDFTCANAFNNSIIPEDTFFPSPESSC

SEQ ID NO: 27 - protein, 241 aa, Artificial Sequence
  Synthetic Construct
GVTQTPRYLIKTRGQQVTLSCSPISGHRSVSWYQQTPGQGLQFLFEYFSETQRNKGNFPGRFSGRQFSNSRSEMNVSTLELGDSALYLCASSFNMATGQYFGPGTRLTVTEDLKNVFPPEVAVFEPSEAEISHTQKATLVCLATGFYPDHVELSWWVNGKEVHSGVCTDPQPLKEQPALNDSRYALSSRLRVSATFWQDPRNHFRCQVQFYGLSENDEWTQDRAKPVTQIVSAEAWGRADC

SEQ ID NO: 28 - protein, 241 aa, Artificial Sequence
  Synthetic Construct
GVTQTPRYLIKTRGQQVTLSCSPISGHRSVSWYQQTPGQGLQFLFEYFSETQRNKGNFPGRFSGRQFSNSRSEMNVSTLELGDSALYLCASSFNMATGQYFGPGTRLTVTEDLKNVFPPEVAVFEPSKAEISRTQKATLVCLATGFYPPHVELSWWVNGKEVHDGVCTDPQPLKEQPALNDSRYALSSRLRVSATFWQDPRNHFRCQVQFYGLSENDEWTQDRAKPVTQIVSAEAWGRADC

SEQ ID NO: 29 - protein, 435 aa, Artificial Sequence
  Synthetic Construct
QEVTQIPAALSVPEGENLVLNCSFTDSAIYNLQWFRQDPGKGLTSLLLISPWQREQTSGRLNASLDKSSGRSTLYIAASQPGDSATYLCAVRPLLDGTYIPTFGRGTSLIVHPYIQNPDPAVYQLRDSKSSDKSVCLFTDFDSQTNVSQSKDSDVYITDKCVLDMRSMDFKSNSAVAWSNKSDFACANAFNNSIIPEDTFFPSPESSCDKTHTCPPCPAPEAAGGPSVFLFPPKPKDTLMISRTPEVTCVVVDVSHEDPEVKFNWYVDGVEVHNAKTKPREEQYQSTYRVVSVLTVLHQDWLNGKEYKCKVSNKALPAPIEKTISKAKGQPREPQVYTLPPSREEMTDNQVSLTCLVKGFYPSDIAVEWESNGQPENNYKTTPPVLMSDGSFFLASKLTVDKSRWQQGNVFSCSVMHEALHNHYTQKSLSLSPGK

SEQ ID NO: 30 - protein, 436 aa, Artificial Sequence
  Synthetic Construct
QEVTQIPAALSVPEGENLVLNCSFTDSAIYNLQWFRQDPGKGLTSLLLISPWQREQTSGRLNASLDKSSGRSTLYIAASQPGDSATYLCAVRPLLDGTYIPTFGRGTSLIVHPYIQNPDPAVYQLRDSKSSDKFVCLFTDFDSQINVSQSKDSDVYITDKCVLDMRSMDFKSNSAVAWSNKSDFTCANAFNNSIIPEDTFFPSPEPKSCDKTHTCPPCPAPEAAGGPSVFLFPPKPKDTLMISRTPEVTCVVVDVSHEDPEVKFNWYVDGVEVHNAKTKPREEQYQSTYRVVSVLTVLHQDWLNGKEYKCKVSNKALPAPIEKTISKAKGQPREPQVYTLPPSREEMTDNQVSLTCLVKGFYPSDIAVEWESNGQPENNYKTTPPVLMSDGSFFLASKLTVDKSRWQQGNVFSCSVMHEALHNHYTQKSLSLSPGK

SEQ ID NO: 31 - protein, 455 aa, Artificial Sequence
  Synthetic Construct
EVQLVESGGGLVQPKGSLKLSCAASGFTFNTYAMNWVRQAPGKGLEWVARIRSKYNNYATYYADSVKDRFTISRDDSQSLLYLQMNNLKTEDTAMYYCVRHGNFGNSYVSWFAYWGQGTLVTVSAASTKGPSVFPLAPSSKSTSGGTAALGCLVADYFPEPVTVSWNSGALTSGVHTFPAVLQSSGLYSLASVVTVPSSSLGTQTYICNVNHKPSNTKVDKRVEPKSCDKTHTCPPCPAPEAAGGPSVFLFPPKPKDTLMISRTPEVTCVVVDVSHEDPEVKFNWYVDGVEVHNAKTKPREEQYQSTYRVVSVLTVLHQDWLNGKEYKCKVSNKALPAPIEKTISKAKGQPRRPRVYTLPPSREEMTKNQVSLVCLVKGFYPSDIAVEWESNGQPENNYKTTPPVLDSDGSFFLYSVLTVDKSRWQQGNVFSCSVMHEALHNHYTQKSLSLSPGK

SEQ ID NO: 32 - protein, 214 aa, Artificial Sequence
  Synthetic Construct
QAVVTQESALTTSPGETVTLTCRSSTGAVTTSNYANWVQEKPDHLFTGLIGGTNKRAPGVPARFSGSLIGDKAALTITGAQTEDEAIYFCALWYSNLWVFGGGTKLTVLGQPKAAPSVTLFPPSSEELQANKATLVCLISDFYPGAVTVAWKADSSPVKAGVETTTPSKQSNNKYAASSYLSLTPEQWKSHRSYSCQVTHEGSTVEKTVAPTEC

SEQ ID NO: 33 - protein, 466 aa, Artificial Sequence
  Synthetic Construct
HHHHHHHHGSQEVTQIPAALSVPEGENLVLNCSFTDSAIYNLQWFRQDPGKGLTSLLLISPWQREQTSGRLNASLDKSSGRSTLYIAASQPGDSATYLCAVRPLLDGTYIPTFGRGTSLIVHPYIQNPDPAVYQLRDSKSSDKFVCLFTDFDSQINVSQSKDSDVYITDKCVLDMRSMDFKSNSAVAWSNKSDFTCANAFNNSIIPEDTFFPSPESSCGGGGSGGGGSGGGGSGGGGSEVQLVESGGGLVQPKGSLKLSCAASGFTFNTYAMNWVRQAPGKGLEWVARIRSKYNNYATYYADSVKDRFTISRDDSQSLLYLQMNNLKTEDTAMYYCVRHGNFGNSYVSWFAYWGQGTLVTVSAASTKGPSVFPLAPCSRSTSESTAALGCLVKDYFPEPVTVSWNSGALTSGVHTFPAVLQSSGLYSLSSVVTVPSSSLGTKTYTCNVDHKPSNTKVDKRVESKYG

SEQ ID NO: 34 - protein, 436 aa, Artificial Sequence
  Synthetic Construct
QEVTQIPAALSVPEGENLVLNCSFTDSAIYNLQWFRQDPGKGLTSLLLISPWQREQTSGRLNASLDKSSGRSTLYIAASQPGDSATYLCAVRPLLDGTYIPTFGRGTSLIVHPYIQNPDPAVYQLRDSKSSDKFVCLFTDFDSQIQVSQSKDSDVYITDKCVLDMRSMDFKSNSAVAWSNKADFTCANAFQNSIIPEDTFFPSPEPKSCDKTHTCPPCPAPEAAGGPSVFLFPPKPKDTLMISRTPEVTCVVVDVSHEDPEVKFNWYVDGVEVHNAKTKPREEQYQSTYRVVSVLTVLHQDWLNGKEYKCKVSNKALPAPIEKTISKAKGQPREPQVYTLPPSREEMTDNQVSLTCLVKGFYPSDIAVEWESNGQPENNYKTTPPVLMSDGSFFLASKLTVDKSRWQQGNVFSCSVMHEALHNHYTQKSLSLSPGK

SEQ ID NO: 35 - protein, 436 aa, Artificial Sequence
  Synthetic Construct
QEVTQIPAALSVPEGENLVLNCSFTDSAIYNLQWFRQDPGKGLTSLLLISPWQREQTSGRLNASLDKSSGRSTLYIAASQPGDSATYLCAVRPFTGGGYIPTFGRGTSLIVHPYIQNPDPAVYQLRDSKSSDKFVCLFTDFDSQINVSQSKDSDVYITDKCVLDMRSMDFKSNSAVAWSNKSDFTCANAFNNSIIPEDTFFPSPEPKSCDKTHTCPPCPAPEAAGGPSVFLFPPKPKDTLMISRTPEVTCVVVDVSHEDPEVKFNWYVDGVEVHNAKTKPREEQYQSTYRVVSVLTVLHQDWLNGKEYKCKVSNKALPAPIEKTISKAKGQPREPQVYTLPPSREEMTDNQVSLTCLVKGFYPSDIAVEWESNGQPENNYKTTPPVLMSDGSFFLASKLTVDKSRWQQGNVFSCSVMHEALHNHYTQKSLSLSPGK

SEQ ID NO: 36 - protein, 242 aa, Artificial Sequence
  Synthetic Construct
GVTQTPKFQVLKTGQSMTLQCAQDMNHEYMSWYRQDPGMGLRLIHYSVAIQTTDQGEVPNGYNVSRSTTEDFPLRLLSAAPSQTSVYFCASSYVGNTGELFFGEGSRLTVLEDLKNVFPPEVAVFEPSKAEISRTQKATLVCLATGFYPPHVELSWWVNGKEVHDGVCTDPQPLKEQPALNDSRYALSSRLRVSATFWQDPRNHFRCQVQFYGLSENDEWTQDRAKPVTQIVSAEAWGRADC

SEQ ID NO: 37 - protein, 436 aa, Artificial Sequence
  Synthetic Construct
QEVTQIPAALSVPEGENLVLNCSFTDSAIYNLQWFRQDPGKGLTSLLLITPWQREQTSGRLNASLDKSSGRSTLYIAASQPGDSATYLCAVRPLLDGTYIPTFGRGTSLIVHPYIQNPDPAVYQLRDSKSSDKFVCLFTDFDSQINVSQSKDSDVYITDKCVLDMRSMDFKSNSAVAWSNKSDFTCANAFNNSIIPEDTFFPSPEPKSCDKTHTCPPCPAPEAAGGPSVFLFPPKPKDTLMISRTPEVTCVVVDVSHEDPEVKFNWYVDGVEVHNAKTKPREEQYQSTYRVVSVLTVLHQDWLNGKEYKCKVSNKALPAPIEKTISKAKGQPREPQVYTLPPSREEMTDNQVSLTCLVKGFYPSDIAVEWESNGQPENNYKTTPPVLMSDGSFFLASKLTVDKSRWQQGNVFSCSVMHEALHNHYTQKSLSLSPGK

SEQ ID NO: 38 - protein, 242 aa, Artificial Sequence
  Synthetic Construct
GVTQTPKFQVLKTGQSMTLQCAQDMNHEYMSWYRQDPGMGLRLIHYSVAIQTTDRGEVPNGYNVSRSTIEDFPLRLLSAAPSQTSVYFCASSYLGNTGELFFGEGSRLTVLEDLKNVFPPEVAVFEPSKAEISRTQKATLVCLATGFYPPHVELSWWVNGKEVHDGVCTDPQPLKEQPALNDSRYALSSRLRVSATFWQDPRNHFRCQVQFYGLSENDEWTQDRAKPVTQIVSAEAWGRADC

SEQ ID NO: 39 - protein, 680 aa, Artificial Sequence
  Synthetic Construct
QEVTQIPAALSVPEGENLVLNCSFTDSAIYNLQWFRQDPGKGLTSLLLISPWQREQTSGRLNASLDKSSGRSTLYIAASQPGDSATYLCAVRPLLDGTYIPTFGRGTSLIVHPYIQNPDPAVYQLRDSKSSDKFVCLFTDFDSQINVSQSKDSDVYITDKCVLDMRSMDFKSNSAVAWSNKSDFTCANAFNNSIIPEDTFFPSPESSCGGGGSGGGGSGGGGSGSEVQLVESGGGLVQPKGSLKLSCAASGFTFNTYAMNWVRQAPGKGLEWVARIRSKYNNYATYYADSVKDRFTISRDDSQSLLYLQMNNLKTEDTAMYYCVRHGNFGNSYVSWFAYWGQGTLVTVSAASTKGPSVFPLAPSSKSTSGGTAALGCLVADYFPEPVTVSWNSGALTSGVHTFPAVLQSSGLYSLASVVTVPSSSLGTQTYICNVNHKPSNTKVDKRVEPKSCDKTHTCPPCPAPEAAGGPSVFLFPPKPKDTLMISRTPEVTCVVVDVSHEDPEVKFNWYVDGVEVHNAKTKPREEQYQSTYRVVSVLTVLHQDWLNGKEYKCKVSNKALPAPIEKTISKAKGQPRRPRVYTLPPSREEMTKNQVSLVCLVKGFYPSDIAVEWESNGQPENNYKTTPPVLDSDGSFFLYSVLTVDKSRWQQGNVFSCSVMHEALHNHYTQKSLSLSPGK

SEQ ID NO: 40 - protein, 470 aa, Artificial Sequence
  Synthetic Construct
HHHHHHHHGSQEVTQIPAALSVPEGENLVLNCSFTDSAIYNLQWFRQDPGKGLTSLLLISPWQREQTSGRLNASLDKSSGRSTLYIAASQPGDSATYLCAVRPLLDGTYIPTFGRGTSLIVHPYIQNPDPAVYQLRDSKSSDKFVCLFTDFDSQINVSQSKDSDVYITDKCVLDMRSMDFKSNSAVAWSNKSDFTCANAFNNSIIPEDTFFPSPESSCGGGGSGGGGSGGGGSGGGGSGGGSEVQLVESGGGLVQPKGSLKLSCAASGFTFNTYAMNWVRQAPGKGLEWVARIRSKYNNYATYYADSVKDRFTISRDDSQSLLYLQMNNLKTEDTAMYYCVRHGNFGNSYVSWFAYWGQGTLVTVSAASTKGPSVFPLAPCSRSTSESTAALGCLVKDYFPEPVTVSWNSGALTSGVHTFPAVLQSSGLYSLSSVVTVPSSSLGTKTYTCNVDHKPSNTKVDKRVESKYG

SEQ ID NO: 41 - protein, 15 aa, Artificial Sequence
  Synthetic Construct
GGGGSGGGGSGGGGS

SEQ ID NO: 42 - protein, 15 aa, Artificial Sequence
  Synthetic Construct
GGGGQGGGGQGGGGQ

SEQ ID NO: 43 - protein, 20 aa, Artificial Sequence
  Synthetic Construct
GGGGSGGGGSGGGGSGGGGS

SEQ ID NO: 44 - protein, 25 aa, Artificial Sequence
  Synthetic Construct
GGGGSGGGGSGGGGSGGGGSGGGGS

SEQ ID NO: 45 - protein, 20 aa, Artificial Sequence
  Synthetic Construct
GGGGQGGGGQGGGGQGGGGQ

SEQ ID NO: 46 - protein, 25 aa, Artificial Sequence
  Synthetic Construct
GGGGQGGGGQGGGGQGGGGQGGGGQ

SEQ ID NO: 47 - protein, 15 aa, Artificial Sequence
  Synthetic Construct
EPKSCDKTHTCPPCP

SEQ ID NO: 48 - protein, 217 aa, Artificial Sequence
  Synthetic Construct
APEAAGGPSVFLFPPKPKDTLMISRTPEVTCVVVDVSHEDPEVKFNWYVDGVEVHNAKTKPREEQYQSTYRVVSVLTVLHQDWLNGKEYKCKVSNKALPAPIEKTISKAKGQPREPQVYTLPPSRDELTKNQVSLTCLVKGFYPSDIAVEWESNGQPENNYKTTPPVLDSDGSFFLYSKLTVDKSRWQQGNVFSCSVMHEALHNHYTQKSLSLSPGK

SEQ ID NO: 49 - protein, 12 aa, Artificial Sequence
  Synthetic Construct
ESKYGPPCPPCP

SEQ ID NO: 50 - protein, 216 aa, Artificial Sequence
  Synthetic Construct
APEAAGGPSVFLFPPKPKDTLMISRTPEVTCVVVDVSQEDPEVQFNWYVDGVEVHNAKTKPREEQFNSTYRVVSVLTVLHQDWLNGKEYKCKVSNKGLPSSIEKTISKAKGQPREPQVYTLPPSQEEMTKNQVSLTCLVKGFYPSDIAVEWESNGQPENNYKTTPPVLDSDGSFFLYSRLTVDKSRWQEGNVFSCSVMHEALHNHYTQKSLSLSLG

SEQ ID NO: 51 - protein, 131 aa, Homo sapiens
EDLKNVFPPEVAVFEPSEAEISHTQKATLVCLATGFYPDHVELSWWVNGKEVHSGVSTDPQPLKEQPALNDSRYCLSSRLRVSATFWQNPRNHFRCQVQFYGLSENDEWTQDRAKPVTQIVSAEAWGRADC

SEQ ID NO: 52 - protein, 95 aa, Homo sapiens
NIQNPDPAVYQLRDSKSSDKSVCLFTDFDSQTNVSQSKDSDVYITDKTVLDMRSMDFKSNSAVAWSNKSDFACANAFNNSIIPEDTFFPSPESSC